European Patent Specification EP 4 043 491 B1, published July 3, 2024. Title: B7-H3 nanobody, preparation method and use thereof. Applicant: DARTSBIOPHARMACEUTICALS LTD.; SHANGHAI MABSTONE BIOTECHNOLOGY LTD.; SHENZHEN INNOVASTONE BIOPHARMA LTD. The sequence listing filed with the application follows.

SEQUENCE LISTING (96 sequences)

SEQ ID NO: 1 - protein, 30 aa, artificial sequence
  FR1
DVQLQESGGGSVQAGGSLRLSCAASGVAHR

SEQ ID NO: 2 - protein, 14 aa, artificial sequence
  FR2
WFRQAPGKEREGVA

SEQ ID NO: 3 - protein, 32 aa, artificial sequence
  FR3
RFTISQDNANDMVYLQMLSLKPEDTAMYYCAA

SEQ ID NO: 4 - protein, 11 aa, artificial sequence
  FR4
WGQGTQVTVSS

SEQ ID NO: 5 - protein, 5 aa, artificial sequence
  CDR1
RYYMS

SEQ ID NO: 6 - protein, 17 aa, artificial sequence
  CDR2
SIYIGSGSTDYVDSVKG

SEQ ID NO: 7 - protein, 14 aa, artificial sequence
  CDR3
GLYGGRWDRAQYKY

SEQ ID NO: 8 - protein, 30 aa, artificial sequence
  FR1
DVQLQESGGGSVQAGGSLRLSCTASGYTRS

SEQ ID NO: 9 - protein, 15 aa, artificial sequence
  FR2
WFRQAPGKEREGVAA

SEQ ID NO: 10 - protein, 35 aa, artificial sequence
  FR3
RFTISQDNAKNAKNTVYLQMNSLKPEDTAMYYCAA

SEQ ID NO: 11 - protein, 11 aa, artificial sequence
  FR4
WGQGTQVTVSS

SEQ ID NO: 12 - protein, 5 aa, artificial sequence
  CDR1
TIWIG

SEQ ID NO: 13 - protein, 16 aa, artificial sequence
  CDR2
IYIGSGATYYVDSVKG

SEQ ID NO: 14 - protein, 19 aa, artificial sequence
  CDR3
TGGTVGSMVRFSPVGDFGY

SEQ ID NO: 15 - protein, 30 aa, artificial sequence
  FR1
DVQLQESGGGLVQPGGSLRLSCAASGFTFT

SEQ ID NO: 16 - protein, 14 aa, artificial sequence
  FR2
WVRQAPGKGLEWVS

SEQ ID NO: 17 - protein, 32 aa, artificial sequence
  FR3
RSTISRDNAKNTLYLQLNSLETEDTAMYYCAK

SEQ ID NO: 18 - protein, 11 aa, artificial sequence
  FR4
RGQGTQVTVSS

SEQ ID NO: 19 - protein, 5 aa, artificial sequence
  CDR1
NYAMS

SEQ ID NO: 20 - protein, 16 aa, artificial sequence
  CDR2
GINSDGGTYYSNSVKG

SEQ ID NO: 21 - protein, 15 aa, artificial sequence
  CDR3
GNGPSWTLGSVDVNS

SEQ ID NO: 22 - protein, 30 aa, artificial sequence
  FR1
DVQLQESGGGSVQAGGSLRLSCAASGDTYR

SEQ ID NO: 23 - protein, 32 aa, artificial sequence
  FR3
RFTISQDSAKNTVYLQMNSLKPEDTAIYYCAA

SEQ ID NO: 24 - protein, 5 aa, artificial sequence
  CDR1
RNTMG

SEQ ID NO: 25 - protein, 17 aa, artificial sequence
  CDR2
AIYTGGTSTAYADSVRG

SEQ ID NO: 26 - protein, 17 aa, artificial sequence
  CDR3
GSVWSRYTWSWPSTYSY

SEQ ID NO: 27 - protein, 30 aa, artificial sequence
  FR1
DVQLQESGGGSVQAGGSLRLSCAASEYSYS

SEQ ID NO: 28 - protein, 32 aa, artificial sequence
  FR3
RFTISQDIAENTVYLRMNSLKPEDTAMYYCAA

SEQ ID NO: 29 - protein, 5 aa, artificial sequence
  CDR1
RKWMG

SEQ ID NO: 30 - protein, 16 aa, artificial sequence
  CDR2
AIYTSGRTAVADSVKG

SEQ ID NO: 31 - protein, 16 aa, artificial sequence
  CDR3
LTGASDSPLRPSEYNY

SEQ ID NO: 32 - protein, 30 aa, artificial sequence
  FR1
DVQLQESGGGSVQAGGSLRLSCAASGFTFS

SEQ ID NO: 33 - protein, 32 aa, artificial sequence
  FR3
RFTISRDNAKNTMYLQMNSLKPEDTAMYYCAA

SEQ ID NO: 34 - protein, 5 aa, artificial sequence
  CDR1
SYDMS

SEQ ID NO: 35 - protein, 17 aa, artificial sequence
  CDR2
AINSGGGSTYYADSVKG

SEQ ID NO: 36 - protein, 21 aa, artificial sequence
  CDR3
DPGSSLAVGAWLKAADPFYGY

SEQ ID NO: 37 - protein, 19 aa, artificial sequence
  CDR3
TSGTVGSMVRFSPVGDFGY

SEQ ID NO: 38 - protein, 30 aa, artificial sequence
  FR1
DVQLQESGGGLVQPGGSLRLSCAASGFTFS

SEQ ID NO: 39 - protein, 14 aa, artificial sequence
  FR2
WVRQAPGRGLEWVS

SEQ ID NO: 40 - protein, 32 aa, artificial sequence
  FR3
RFTISRDNAKKMLYLQMDSLKPEDTAVYYCAT

SEQ ID NO: 41 - protein, 5 aa, artificial sequence
  CDR1
GVDMS

SEQ ID NO: 42 - protein, 17 aa, artificial sequence
  CDR2
GFGSGGESPSYADSVKG

SEQ ID NO: 43 - protein, 6 aa, artificial sequence
  CDR3
RWAEGY

SEQ ID NO: 44 - protein, 30 aa, artificial sequence
  FR1
DVQLQESGGGLVQPGGSLRLSCAASGFLFS

SEQ ID NO: 45 - protein, 32 aa, artificial sequence
  FR3
RFTISRDNAKNTLTLQLNSLKTEDTAMYYCAK

SEQ ID NO: 46 - protein, 5 aa, artificial sequence
  CDR1
RYSMS

SEQ ID NO: 47 - protein, 17 aa, artificial sequence
  CDR2
GITNGGSITKYADSVKG

SEQ ID NO: 48 - protein, 15 aa, artificial sequence
  CDR3
GAGEYGPVSDYVFSL

SEQ ID NO: 49 - protein, 30 aa, artificial sequence
  FR1
DVQLQESGGGSVQAGGSLRLSCAASGYTIG

SEQ ID NO: 50 - protein, 32 aa, artificial sequence
  FR3
RFAISEDNAKNTVYLHMNLLKPEDTAMYYCAA

SEQ ID NO: 51 - protein, 5 aa, artificial sequence
  CDR1
SNYMG

SEQ ID NO: 52 - protein, 17 aa, artificial sequence
  CDR2
AIYTGGGNTYYADSVKG

SEQ ID NO: 53 - protein, 16 aa, artificial sequence
  CDR3
DLRLRVAVLHPYGYNY

SEQ ID NO: 54 - protein, 30 aa, artificial sequence
  FR1
DVQLQESGGGLVQPGGSLRLSCAVSGFTFS

SEQ ID NO: 55 - protein, 15 aa, artificial sequence
  FR2
SWVRQAPGKGLEWVS

SEQ ID NO: 56 - protein, 32 aa, artificial sequence
  FR3
RFTISRDNAKNTLYLQLNNLKTEDTAMYYCTK

SEQ ID NO: 57 - protein, 11 aa, artificial sequence
  FR4
GGQGTQVTVSS

SEQ ID NO: 58 - protein, 4 aa, artificial sequence
  CDR1
NYAM

SEQ ID NO: 59 - protein, 16 aa, artificial sequence
  CDR2
RISSSGITYYADSVKG

SEQ ID NO: 60 - protein, 5 aa, artificial sequence
  CDR3
SSEAP

SEQ ID NO: 61 - protein, 30 aa, artificial sequence
  FR1
DVQLQESGGGSVQAGGSLRLSCAASGAIYR

SEQ ID NO: 62 - protein, 32 aa, artificial sequence
  FR3
RFTISQDNAKNTVYLQMNDLKPEDTAMYYCAA

SEQ ID NO: 63 - protein, 5 aa, artificial sequence
  CDR1
GNYMG

SEQ ID NO: 64 - protein, 17 aa, artificial sequence
  CDR2
AIATNGRTTYYADSVKG

SEQ ID NO: 65 - protein, 19 aa, artificial sequence
  CDR3
DNSWSCTVVGGLLAPAYNY

SEQ ID NO: 66 - protein, 30 aa, artificial sequence
  FR1
DVQLQESGGGSVQAGGSLRLSCAASRFTYS

SEQ ID NO: 67 - protein, 32 aa, artificial sequence
  FR3
RFTISLDIAKKTLSLQMDSLKSEDTAMYYCAA

SEQ ID NO: 68 - protein, 5 aa, artificial sequence
  CDR1
WYCMG

SEQ ID NO: 69 - protein, 17 aa, artificial sequence
  CDR2
AICTTPSRTYAADSVKG

SEQ ID NO: 70 - protein, 18 aa, artificial sequence
  CDR3
DTRGAIGFFKGSGPAIPY

SEQ ID NO: 71 - protein, 123 aa, artificial sequence
  No. 1 nanobody
DVQLQESGGGSVQAGGSLRLSCAASGVAHRRYYMSWFRQAPGKEREGVASIYIGSGSTDYVDSVKGRFTISQDNANDMVYLQMLSLKPEDTAMYYCAAGLYGGRWDRAQYKYWGQGTQVTVSS

SEQ ID NO: 72 - protein, 131 aa, artificial sequence
  No. 2 nanobody
DVQLQESGGGSVQAGGSLRLSCTASGYTRSTIWIGWFRQAPGKEREGVAAIYIGSGATYYVDSVKGRFTISQDNAKNAKNTVYLQMNSLKPEDTAMYYCAATGGTVGSMVRFSPVGDFGYWGQGTQVTVSS

SEQ ID NO: 73 - protein, 123 aa, artificial sequence
  No. 3 nanobody
DVQLQESGGGLVQPGGSLRLSCAASGFTFTNYAMSWVRQAPGKGLEWVSGINSDGGTYYSNSVKGRSTISRDNAKNTLYLQLNSLETEDTAMYYCAKGNGPSWTLGSVDVNSRGQGTQVTVSS

SEQ ID NO: 74 - protein, 126 aa, artificial sequence
  No. 4 nanobody
DVQLQESGGGSVQAGGSLRLSCAASGDTYRRNTMGWFRQAPGKEREGVAAIYTGGTSTAYADSVRGRFTISQDSAKNTVYLQMNSLKPEDTAIYYCAAGSVWSRYTWSWPSTYSYWGQGTQVTVSS

SEQ ID NO: 75 - protein, 124 aa, artificial sequence
  No. 5 nanobody
DVQLQESGGGSVQAGGSLRLSCAASEYSYSRKWMGWFRQAPGKEREGVAAIYTSGRTAVADSVKGRFTISQDIAENTVYLRMNSLKPEDTAMYYCAALTGASDSPLRPSEYNYWGQGTQVTVSS

SEQ ID NO: 76 - protein, 130 aa, artificial sequence
  No. 6 nanobody
DVQLQESGGGSVQAGGSLRLSCAASGFTFSSYDMSWVRQAPGKGLEWVSAINSGGGSTYYADSVKGRFTISRDNAKNTMYLQMNSLKPEDTAMYYCAADPGSSLAVGAWLKAADPFYGYWGQGTQVTVSS

SEQ ID NO: 77 - protein, 131 aa, artificial sequence
  No. 7 nanobody
DVQLQESGGGSVQAGGSLRLSCTASGYTRSTIWIGWFRQAPGKEREGVAAIYIGSGATYYVDSVKGRFTISQDNAKNAKNTVYLQMNSLKPEDTAMYYCAATSGTVGSMVRFSPVGDFGYWGQGTQVTVSS

SEQ ID NO: 78 - protein, 115 aa, artificial sequence
  No. 8 nanobody
DVQLQESGGGLVQPGGSLRLSCAASGFTFSGVDMSWVRQAPGRGLEWVSGFGSGGESPSYADSVKGRFTISRDNAKKMLYLQMDSLKPEDTAVYYCATRWAEGYWGQGTQVTVSS

SEQ ID NO: 79 - protein, 124 aa, artificial sequence
  No. 9 nanobody
DVQLQESGGGLVQPGGSLRLSCAASGFLFSRYSMSWVRQAPGKGLEWVSGITNGGSITKYADSVKGRFTISRDNAKNTLTLQLNSLKTEDTAMYYCAKGAGEYGPVSDYVFSLRGQGTQVTVSS

SEQ ID NO: 80 - protein, 125 aa, artificial sequence
  No. 10 nanobody
DVQLQESGGGSVQAGGSLRLSCAASGYTIGSNYMGWFRQAPGKEREGVAAIYTGGGNTYYADSVKGRFAISEDNAKNTVYLHMNLLKPEDTAMYYCAADLRLRVAVLHPYGYNYWGQGTQVTVSS

SEQ ID NO: 81 - protein, 113 aa, artificial sequence
  No. 11 nanobody
DVQLQESGGGLVQPGGSLRLSCAVSGFTFSNYAMSWVRQAPGKGLEWVSRISSSGITYYADSVKGRFTISRDNAKNTLYLQLNNLKTEDTAMYYCTKSSEAPGGQGTQVTVSS

SEQ ID NO: 82 - protein, 128 aa, artificial sequence
  No. 12 nanobody
DVQLQESGGGSVQAGGSLRLSCAASGAIYRGNYMGWFRQAPGKEREGVAAIATNGRTTYYADSVKGRFTISQDNAKNTVYLQMNDLKPEDTAMYYCAADNSWSCTVVGGLLAPAYNYWGQGTQVTVSS

SEQ ID NO: 83 - protein, 127 aa, artificial sequence
  No. 13 nanobody
DVQLQESGGGSVQAGGSLRLSCAASRFTYSWYCMGWFRQAPGKEREGVAAICTTPSRTYAADSVKGRFTISLDIAKKTLSLQMDSLKSEDTAMYYCAADTRGAIGFFKGSGPAIPYWGQGTQVTVSS

SEQ ID NO: 84 - DNA, 369 bp, artificial sequence
  DNA of No. 1 nanobody
gatgtgcagctgcaggagtctggaggaggctcggtgcaggctggagggtctctgagactctcctgtgcagcctctggtgtcgcccacaggcgctactacatgtcctggttccgccaggctccagggaaggagcgcgagggggtcgcatccatttatattggtagtggtagcacagactatgtcgactccgtgaagggccgattcaccatctcccaagacaacgccaacgacatggtgtatctgcaaatgctcagcctcaaacctgaggacactgccatgtactactgtgcggcaggcctttacggtggtagatgggatcgggcccagtataagtactggggccaggggacccaggtcaccgtctcctca

SEQ ID NO: 85 - DNA, 393 bp, artificial sequence
  DNA of No. 2 nanobody
gatgtgcagctgcaggagtctggaggaggctcggtgcaggctggagggtctctgagactctcctgtacagcctccggatacacccgcagtaccatttggataggctggttccgccaggctccagggaaggagcgcgagggggtcgcagctatttatattggtagtggcgcgacatactatgtggactccgtgaagggccgattcaccatctcccaagacaacgccaagaacgccaagaacacggtgtatctgcagatgaacagcctgaaacctgaggacactgccatgtactactgtgcggcaacgggcggtactgtaggaagtatggtccgattctccccagtgggcgactttggttattggggccaggggacccaggtcaccgtctcctca

SEQ ID NO: 86 - DNA, 369 bp, artificial sequence
  DNA of No. 3 nanobody
gatgtgcagctgcaggagtctggaggaggcttggtgcagcctggggggtctctgagactctcctgtgcagcctctggattcaccttcacaaactatgccatgagctgggtccgccaggctccagggaagggactcgagtgggtctcaggtattaatagtgatggtggcacatactattcaaactccgtgaagggccgaagcaccatctccagagacaacgccaagaacacgctgtatctgcaattgaacagcctggagactgaggacacggccatgtattactgtgcaaaaggaaacggcccgtcttggaccctggggagcgtggacgttaactcccggggccaggggacccaggtcaccgtctcctca

SEQ ID NO: 87 - DNA, 378 bp, artificial sequence
  DNA of No. 4 nanobody
gatgtgcagctgcaggagtctggaggaggctcggtgcaggctggagggtctctgagactctcctgtgcagcctctggagacacttacaggcgcaacaccatgggctggttccgccaggctccggggaaggagcgcgagggggtcgcagctatttatactggtggtactagtacagcctatgccgactccgtgaggggccgattcaccatctcccaagacagcgccaagaacacggtgtatctgcaaatgaacagcctgaaacctgaggacactgccatatactactgtgcggcaggctcagtgtggtcccgttatacatggtcctggcccagtacgtatagctactggggccaggggacccaggtcaccgtctcctca

SEQ ID NO: 88 - DNA, 372 bp, artificial sequence
  DNA of No. 5 nanobody
gatgtgcagctgcaggagtctggaggaggctcggtgcaggctggagggtctctgagactctcctgtgcagcctctgaatacagctacagtaggaagtggatgggctggttccgccaggctccagggaaggagcgcgagggggtcgcagctatttatactagtggtaggacagccgttgccgactccgtgaagggccgattcaccatctcccaagacatcgccgagaacacggtgtatctgcgtatgaacagcctgaaacctgaggacactgccatgtactactgtgcggcactcacaggtgctagcgactcaccgctacgcccaagcgagtataactactggggccaggggacccaggtcaccgtctcctca

SEQ ID NO: 89 - DNA, 390 bp, artificial sequence
  DNA of No. 6 nanobody
gatgtgcagctgcaggagtctggaggaggctcggtgcaggctggagggtctctgagactctcctgtgcagcctctggattcacattcagtagctacgacatgagctgggtccgccaggctccagggaaggggctcgagtgggtctcagctattaatagtggtggtggtagcacatactatgcagactccgtgaagggccgattcaccatctccagagacaacgccaagaacacgatgtatctgcaaatgaacagcctgaaacctgaggacactgccatgtactactgtgcggcagatcctggttcaagtttggcggtgggagcttggttgaaggcggcggatcccttctatggttactggggccaggggacccaggtcaccgtctcctca

SEQ ID NO: 90 - DNA, 393 bp, artificial sequence
  DNA of No. 7 nanobody
gatgtgcagctgcaggagtctggaggaggctcggtgcaggctggagggtctctgagactctcctgtacagcctccggatacacccgcagtaccatttggataggctggttccgccaggctccagggaaggagcgcgagggggtcgcagctatttatattggtagtggcgcgacatactatgtggactccgtgaagggccgattcaccatctcccaagacaacgccaagaacgccaagaacacggtgtatctgcagatgaacagcctgaaacctgaggacactgccatgtactactgtgcggcaacgagcggtactgtaggaagtatggtccgattctccccagtgggcgactttggttattggggccaggggacccaggtcaccgtctcctca

SEQ ID NO: 91 - DNA, 345 bp, artificial sequence
  DNA of No. 8 nanobody
gatgtgcagctgcaggagtctggaggaggcttggtgcagcctggggggtctctgagactctcctgtgcagcctctggattcacattcagtggcgtcgacatgagctgggtccgccaggctccagggagggggctcgagtgggtctcagggtttggtagtggtggtgaaagcccatcatatgcagactccgtgaagggccgattcaccatctccagagacaacgccaagaaaatgctgtatctgcagatggacagtttgaaacctgaggacacagccgtgtattactgcgccacccgctgggctgagggctactggggccaggggacccaggtcaccgtctcctca

SEQ ID NO: 92 - DNA, 372 bp, artificial sequence
  DNA of No. 9 nanobody
gatgtgcagctgcaggagtctggaggaggcttggtgcagcctggggggtctctgagactctcctgtgcagcctctggattcctcttcagtagatattccatgagttgggtccgccaggctccagggaagggactcgagtgggtctcaggtattacgaatggtggtagcattacaaagtatgcagactccgtgaagggccgattcaccatctccagagacaacgccaagaacacactgactctgcaactgaacagcctgaaaactgaggacacggccatgtattactgtgccaaaggcgcgggggagtatggccctgttagtgactatgtcttctctctcaggggccaggggacccaggtcaccgtctcctca

SEQ ID NO: 93 - DNA, 375 bp, artificial sequence
  DNA of No. 10 nanobody
gatgtgcagctgcaggagtctggaggaggctcggtgcaggctggagggtctctgagactctcctgtgcagcctctggatacaccatcggtagcaactacatgggctggttccgccaggctccagggaaggagcgcgagggggtcgcagctatttatactggtggtggtaatacatactatgccgactccgtgaagggccgattcgccatctccgaagacaacgccaagaacacggtgtatctgcacatgaacctcctgaaacctgaggacactgccatgtactactgtgcggcagacttgagactacgggttgctgtactccacccgtatgggtataactactggggccaggggacccaggtcaccgtctcctca

SEQ ID NO: 94 - DNA, 339 bp, artificial sequence
  DNA of No. 11 nanobody
gatgtgcagctgcaggagtctggaggaggcttggtgcagcctggggggtctctgagactctcctgtgcagtctctggattcaccttcagtaactatgccatgagctgggtccgccaggctccagggaaggggctcgagtgggtctcacgtattagtagtagtggtattacatactatgcagactccgtgaagggccgattcaccatctccagagacaacgccaagaacacgctgtatctacaattgaacaacctgaaaactgaggacacggccatgtattactgtacaaaaagttccgaggccccgggtggccaggggacccaggtcaccgtctcctca

SEQ ID NO: 95 - DNA, 384 bp, artificial sequence
  DNA of No. 12 nanobody
gatgtgcagctgcaggagtctggaggaggctcggtacaggctggagggtctctgagactctcctgtgcagcctctggagccatctacagaggcaactacatgggctggttccgccaggctccagggaaggagcgcgagggggtcgcggctatcgctactaatggtcgtacaacatactatgccgactccgtgaagggccgattcaccatctcccaagacaacgccaagaacacggtgtatctgcaaatgaacgacctgaaacctgaggacactgccatgtactactgtgcggcagacaactcttggtcctgtacggtggtaggtgggctactggcgcctgcctataactactggggccaggggacccaggtcaccgtctcctca

SEQ ID NO: 96 - DNA, 381 bp, artificial sequence
  DNA of No. 13 nanobody
gatgtgcagctgcaggagtctggaggaggctcggtgcaggctggagggtctctgagactctcctgtgcagcctctagatttacctacagttggtactgcatgggctggttccgccaggctccggggaaggagcgcgagggggtcgcagctatttgcacgacaccgagccgcacatacgctgccgactccgtgaagggtcgattcaccatctccctagacatcgccaagaagacgctgtctctgcaaatggacagcctgaaatctgaggacactgccatgtactactgtgcggcagatacaagaggagctatagggttcttcaagggcagtgggcccgccatcccctactggggccaggggacccaggtcaccgtctcctca